European Patent Application EP 4 717 778 A2, published April 1, 2026. Title: IMMUNOGENIC COMPOSITION. Applicant: GlaxoSmithKline Biologicals SA. The sequence listing filed with the application follows.

SEQUENCE LISTING (66 sequences)

SEQ ID NO: 1 - skipped

SEQ ID NO: 2 - protein, 5 aa, synthetic construct
  REGION 1..5: note = consensus sequence
DQNAT

SEQ ID NO: 3 - skipped

SEQ ID NO: 4 - protein, 7 aa, synthetic construct
  REGION 1..7: note = consensus sequence
KDQNATK

SEQ ID NO: 5 - protein, 481 aa, Streptococcus pneumoniae
MSRRFKKSGSQKVKRSVNIVLLTIYLLLVCFLLFLIFKYNILAFRYLNLVVTALVLLVALVGLLLIIYKKAEKFTIFLLVFSILVSSVSLFAVQQFVGLTNRLNATSNYSEYSISVAVLADSDIENVTQLTSVTAPTGTDNENIQKLLADIKSSQNTDLTVNQSSSYLAAYKSLIAGETKAIVLNSVFENIIESEYPDYASKIKKIYTKGFTKKVEAPKTSKNQSFNIYVSGIDTYGPISSVSRSDVNILMTVNRDTKKILLTTTPRDAYVPIADGGNNQKDKLTHAGIYGVDSSIHTLENLYGVDINYYVRLNFTSFLKLIDLLGGIDVYNDQEFTAHTNGKYYPAGNVHLDSEQALGFVRERYSLADGDRDRGRNQQKVIVAILQKLTSTEALKNYSTIINSLQDSIQTNMPLETMINLVNAQLESGGNYKVNSQDLKGTGRTDLPSYAMPDSNLYVMEIDDSSLAVVKAAIQDVMEGR

SEQ ID NO: 6 - protein, 243 aa, Streptococcus pneumoniae
MIDIHSHIVFDVDDGPKSREESKALLTESYRQGVRTIVSTSHRRKGMFETPEEKIAENFLQVREIAKEVADDLVIAYGAEIYYTLDALEKLEKKEIPTLNDSRYALIEFSMNTPYRDIHSALSKILMLGITPVIAHIERYDALENNGKRVRELIDMGCYTQINSYHVSKPKFFGEKYKFMKKRARYFLERDLVHVVASDMHNLDSRPPYMQQAYDIIAKKYGAKKAKELFVDNPRKIIMDQLI

SEQ ID NO: 7 - protein, 230 aa, Streptococcus pneumoniae
MKEQNTLEIDVLQLFRALWKRKLVILLVAIITSSVAFTYSTFVIKPEFTSTTRIYVVNRNQGEKSGLTNQDLQAGTYLVKDYREIILSQDVLEEVVSDLKLDLTPKGLANKIKVTVPVDTRIVSVSVNDRVPEEASRIANSLREVAAQKIISITRVSDVTTLEEARPAISPSSPNIKRNILIGFLAGVIGTSVIVLLLELLDTRVKRPEDIEDTLQMTLLGVVPNLNKLK

SEQ ID NO: 8 - protein, 227 aa, Streptococcus pneumoniae
MPTLEIAQKKLEFIKKAEEYYNALCTNIQLSGDKLKVISVTSVSPGEGKTTTSVNIAWSFARAGYKTLLIDGDTRNSVISGFFKSREKITGLTEFLSGTADLSHGLCDTNIENLFVVQSGSVSPNPTALLQSKNFNDMIETLRKYFDYIIVDTAPIGIVIDAAIITQKCDASILVTATGEANKRDVQKAKQQLKQTGKLFLGVVLNKLDISVDKYGVYGFYGNYGKK

SEQ ID NO: 9 - protein, 455 aa, Streptococcus pneumoniae
MDEKGLKIFMAVLQSIIVILLVYFLSFVRETELERSSMVILYLLHFFVFYVSSYGNNFFKRGYLVEFNSTIRYIFFFAIAISVLNFFIAERFSISRRGMVYFLTLEGISLYLLNFLVKKYWKHVFFNLKNSKKILLLTVTKNMEKVLDKLLESDELSWKLVAVSVLNKSDFQHDKIPVIEKEKIIEFATHEVVDEVFVNLPGESYDIGEIISRFETMGIDVTVNLKAFDKNLGRNKQIHEMVGLNVVTFSTNFYKTSHVISKRILDICGATIGLILFAIASLVLVPLIRKDGGPAIFAQTRIGKNGRHFTFYKFRSMRIDAEAIKEQLMDQNTMQGGMFKIDNDPRVTKIGRFIRKTSLDELPQFWNVFIGDMSLVGTRPPTVDEYDQYTPEQKRRLSFKPGITGLWQVSGRSKITDFDDVVKLDVSYIDNWTIWKDIEILLKTVKVVFMRDGAK

SEQ ID NO: 10 - protein, 392 aa, Streptococcus pneumoniae
MKKSVYIIGSKGIPAKYGGFETFVEKLTAFQQDKAIQYYVACMRENSAKSGTTEDVFEHNGAICYNVDVPNIGPARAIVYDIAAINRAIEIAKENKDEDPIFYILACRIGPFIHGIKKKIQAIGGTLLVNPDGHEWLRAKWSTPVRRYWKISEGLMVKHADLLVCDSKNIEQYIQEDYKQFQPKTTYIAYGTDTTRSILKSSDEKVRSWFKEKNVSENEYYLVVGRFVPENNYESMILGFLASNSKKDFVLITNVEQNKFYNQLLAKTGFDKDPRVKFVGTVYNQELLKYIRENAFAYFHGHEVGGTNPSLLEALASTKLNLLLDVGFNREVAEDGADYWEKDNLHKVIEASEQKTQEEINEKNILSTKQVTERFSWDLIVNEYEKLFTRKN

SEQ ID NO: 11 - protein, 468 aa, Streptococcus pneumoniae
MRYGIMRISFSKKTMLCGLLYIGLILSVVTIPTIVTFLYSLLFIGIVTVLNYNSILASDEDANSFFVALPIILSSFQNVYLGFGADRLNSVTLQVLLSISIAIITITVFLGIILNRFKSKEFSWLVLSILVIIIQSVILLIFFPTTLPAYLSSMRNILAPLLIFYFSIYGFKNINLQKFYKYMFIIILVVLIFGFIEYIYGNSLWTRLNIKKLWALKGLAIENRVVPGNWHSSELIGGKQLRRMVSTFADPVNLGSYLFAAFMLAWYKNKKLLQVLLLASFVLSVSKAAFLSMLVYIIIYTWVVDKNKILSIFGIIISTVLGLYFYNFSQVSSYGSINAHIDGFFSALSTPLHYPFGMGVGSVGVLASKLGSQTALSSEVLETGIGMIIAQLGFVGVIIYLIFFVKLSVIGKNINNKRDKILWFTLIYSFLANAFFNEVALSPNSCTLYFLILGLLYNKNKIRSTEFS

SEQ ID NO: 12 - protein, 323 aa, Streptococcus pneumoniae
MEKLVSIILPVYNVEQYIKNCLESIQQQTYPNLEVIIVNDGSTDKSVEYCEQICKIDSRFSITHKENGGLSDARNVGIDKAKGDYLIFVDSDDFVSQDMVSYLVSCMENNEADIAICDPVHYYSDRQNNDLNIFSPASSVKVYETTEALCEMFYQKSFLVSAWAKIFKRELFDDIRFPVGKLFEDSAIMYLLLEKCETIAYSDAKLYAYVHRDNSITTKKFSDRDLDILEITNTIINHYGDNLRVYTAAVSYKVSACFRILLNSPSEEKYKKVQKECLSYILQNWRNILFNNNVRLKNKLALISITIFNPFVKLIYSKVNRWE

SEQ ID NO: 13 - protein, 410 aa, Streptococcus pneumoniae
MNKYEERYQENLSKNDFYKLINKSYLSDKELQVQQVKAGIVLPPKAFETKLSNKLGLQKSLHGKGGVVDSNGNYIELSAQKAVGMRNRVYGPYKINYDNLPIRNEKVIYLNYFIKQWGHFLLDVVGRLWYPLLQDNDTKLVYTCYAGTETKIEGNYLEFLKLLGIDQSRLIMINCPTQFSEVIIPESSILPGGYYTKEYKQLFSSVVENIKLDKYDVNAKMIYCSRSKLGIAKSKEFGEDGIEGIFKQNGYTSVYMETMSLEEQIKTLLSAKTIVLTSGSLAHNLLFVNKDIDVFILNKTYRVNLHQFLINEISDATVRFVDIYRSPLPILYGYGPFLMDLTKPLANFLDDNEFVYEKGTVLSKKDYFKYYLKWLWSYRFFLFRLNGIKEGNSEFEKSFKIIRRYYKTGR

SEQ ID NO: 14 - protein, 461 aa, Streptococcus pneumoniae
MSKYKELAKNTGIFALANFSSKILIFLLVPIYTRVLTTTEYGFYDLVYTTIQLFVPILTLNISEAVMRFLMKDGVSKKSVFSIAVLDIFIGSIAFALLLLVNNLFSLSDLISQYSIYIFVIFVFYTLNNFLIQFSKGIDKIGVTAISGVISTAVMLAMNVILLVVFDWGLLGFFIANVCGYVIPCIYIVSRLRLWELFEIKIDKKLQWEMVYYALPLVLNILSWWVNNTSDRYIVTAIVGIQASAIISVAYKIPQILSTISAIFIQSWQISAIKIQEDKSGTTFVSNMLLYYNALLLIIASGIILFVKPISNILFGISFYSAWELVPFLIISSLFNAISGCIGAIMGAKMDTHNIAKSALVGMIANIILNIVLTFLMGPQGITISTLIASFLIFYMRKDSVKEINSETYRAIYLSWILLVVEACLLIYMDFIIGALIAMVINLFLLKDVIKPLYLKIFKRN

SEQ ID NO: 15 - protein, 382 aa, Streptococcus pneumoniae
MIVLQYFKILARFVFMFLISAVLLPFKIKPNKIVFINFNGKGYGDNPKSICEYLRTTYPDLDLVWLARDNEGFPDGVRVVKYGTFQAFYEQASSKVWVYNVRAFARILKKRGQIYIQTWHGASSFKLIEKQADLPINYVLEAKYDARVTDIMISDSRKQTEEFQKYFWYSGEIFEVGMPRNDALFHYKEDYDKLNNIRKELSIHSDDYVILYAPTFRDDGDASYLDINFERLLQCVEHGIKKKCKFLIRLHPNHSHLCNNISFNKNIINATFYSDMQELTLLADVLVTDYSSSIFDFMLLNKPYVRYVNDLEKYAELRGVSDTYYELPDSIIKTAEELYDLLPKKIENFDYDSIKKYRNEILCPIFNGTASENVGRRIIQEL

SEQ ID NO: 16 - protein, 342 aa, Streptococcus pneumoniae
MKNNDLKIGSGAIHQISATLSQNSISGKILYCADPVVDDLYGSIVRSQIEEIGRVKEESCNYNTIAYAMNIAERAIATDIDCIVGMGGGRVLDVCKYASFISKRPYLSIPTTAANDGIASPVAVLKRQDDRPKSLGAAIPSMTLIDIDVIASGPIQNIKAGIGDTISNYTALKDWELAVERGKDEMHGFAYLMSQNSLDALMKTKYNSITPDFIEVLVNSLVLSGIAMDFAGSSRPVSGSEHLFSHALDYYGSTRNLHGIQVALGTVAVLKLIENSVDTVVDYLQRFEVHINPKLLGIDEELFIYCMQHATKMRSNRYTYLHEVDLSTDRLKQIYKELISEL

SEQ ID NO: 17 - protein, 234 aa, Streptococcus pneumoniae
MKALILAAGLGTRLAPITNEVPKSLVPVNGKPILMKQIENLYQNNITDITIIAGYKSSVLTDAVTEKYPEINIIDNVDFKTTNNMYSAYLGKAAMGDSDFLMMNADVFYDASVIKSLLLHKAPNAIVTDLGIYIEESMKVVEKNGRLVEISKQISPEETLGASIDVYKFSYEAGARFFEKCKEFIEDKRELQMWSEVALNAILSEVEFVACPLEGRWLEIDNHEDLVAAEKLFA

SEQ ID NO: 18 - protein, 277 aa, Streptococcus pneumoniae
MKLTNRVDYFGADISELQNKKLFLFDMDGTIYEEDRLFEGTLELLDYIHNIGGEYIFITNNSSKSVVDYVEKVNRLGIKAERDNFFTSAQATIVYIKENYPKSKVYCQGTKSLIKELSDAGIDVTEQVSADIDVVLVGFDTELTSDKIRNTCEILSTKDVPFIATNPDIRCPVSFGFIPDCGSICDMISKSVDRKPVYIGKPEPTMVDIVRKKLNYSLFETVVIGDRLYTDIMTGINAGVTSVCVLTGEATVNDIQQDSIKPTYTFKNVKEMWKGIV

SEQ ID NO: 19 - protein, 289 aa, Streptococcus pneumoniae
MKGIILAGGSGTRLYPLTRAASKQLMPVYDKPMIYYPLSTLMLAGIRDILIISTPQDLPRFKELLQDGSEFGIKLSYAEQPSPDGLAQAFIIGEEFIGDDSVALILGDNIYHGPGLSTMLQKAAKKEKGATVFGYHVKDPERFGVVEFDENMNAISIEEKPEYPRSNYAVTGLYFYDNDVVEIAKSIKPSPRGELEITDVNKAYLDRGDLSVELMGRGFAWLDTGTHESLLEASQYIETVQRMQNVQVANLEEIAYRRGYISREDVLALAQSLKKNEYGQYLLRLIGEA

SEQ ID NO: 20 - protein, 197 aa, Streptococcus pneumoniae
MTDNFFGKTLAARKVEAIPGMLEFDIPVHGDNRGWFKENFQKEKMLPLGFPESFFAEGKLQNNVSFSRKNVLRGLHAEPWDKYISVADGGKVLGSWVDLREGETFGNTYQTVIDASKGIFVPRGVANGFQVLSDTVSYSYLVNDYWALELKPKYAFVNYADPSLGIEWENIAEAEVSEADKNHPLLKDVKPLKKEDL

SEQ ID NO: 21 - protein, 349 aa, Streptococcus pneumoniae
MTEYKNIIVTGGAGFIGSNFVHYVYENFPDVHVTVLDKLTYAGNRANIEEILGNRVELVVGDIADAELVDKLAAQADAIVHYAAESHNDNSLNDPSPFIHTNFIGTYTLLEAARKYDIRFHHVSTDEVYGDLPLREDLPGHGEGPGEKFTAETKYNPSSPYSSTKAASDLIVKAWVRSFGVKATISNCSNNYGPYQHIEKFIPRQITNILSGIKPKLYGEGKNVRDWIHTNDHSSGVWTILTKGQIGETYLIGADGEKNNKEVLELILKEMGQAVDAYDHVTDRAGHDLRYAIDASKLRDELGWKPEFTNFEAGLKATIKWYTDNQEWWKAEKEAVEANYAKTQEIITV

SEQ ID NO: 22 - protein, 283 aa, Streptococcus pneumoniae
MILITGANGQLGTELRYLLDERNEEYVAVDVAEMDITDAEMVEKVFEEVKPTLVYHCAAYTAVDAAEDEGRELDFAINVTGTKNVAKASEKHGATLVYISTDYVFDGKKPVGQEWEVDDRPDPQTEYGRTKRMGEELVEKHVSNFYIIRTAWVFGNYGKNFVFTMQNLAKTHKTLTVVNDQYGRPTWTRTLAEFMTYLAENRKEFGYYHLSNDATEDTTWYDFAVEILKGTDVEVKPVDSSQFPAKAKRPLNSTMSLAKAKATGFVIPTWQDALQEFYKQEVR

SEQ ID NO: 23 - protein, 484 aa, Streptococcus pneumoniae
MLIMSRRFKKSGSQKVKRSVNIVLLTIYLLLVCFLLFLIFKYNILAFRYFNLVVTALVLLVALVGLLLIIYKKAEKFTIFLLVFSILVSSVSLFAVQQFVGLTNRLNATSNYSEYSISVAVLADSDIENVTQLTSVTAPTGTDNENIQKLLADIKSSQNIDLTVNQSSSYLAAYKSLIAGETKAIVLNSVFENIIESEYPDYASKIKKIYTKGFTKKVEAPKTSKNQSFNIYVSGIDTYGPISSVSRSDVNILMTVNRDTKKILLTTTPRDAYVPIADGGNNQKDKLTHAGIYGVDSSIHTLENLYGVDIHYYVRLNFTSFLKLIDLLGGVDVYNDQDFTSLHGKFHFPVGNVHLDSEQALGFVRERYSLADGDHDRGRNQQKVIAAILQKLTSSEALKNYSMIIDSLQDSIQTNMPLETMINLVNAQLESGGTYKVNSQDLKGRGRTDLPSYAMPDSNLYMMEINDSSLASVKTAIQDVLEGR

SEQ ID NO: 24 - protein, 259 aa, Streptococcus pneumoniae
MHLSKLLFRMCWRADEMIDIHSHIVFDVDDGPKSREESKALLTEAYRQGVRTIVSTSHRRKGMFETPEEKIAENFLQVREIAKEVASDLVIAYGAEIYYTPDVLGKLEKNRIPTLNNSRYALIEFSMNTPYRDIHSALIKILMLGITPVIAHIERYDALENNEKRVRELINMGCYTQVNSSHVLKSKLFGEPYKFMKKRAQYFLERDLVHVIASDMHNVDSRPPHMAEAYDLVSQKYGETKAQDLFIDNPRKIVMDQLI

SEQ ID NO: 25 - protein, 230 aa, Streptococcus pneumoniae
MKEQNTIEIDVFQLLKTLWKHKLIILLVALVTGAGAFAYSIFIVKPEYTSTTRIYVVNRNQENKPGLTNQDLQAGTYLVKDYHEIILSQDVLEKVATNLKLDIPVKTLTSKVQVTVPADTRIVSISVKDKQPEEASRIANSIREVAAEKIIAVTRVSDVTTLEEARPATTPSSPNVRRNTLVGFLGAAAVTVITVLLIELFDTRVKRPEEVEDVLQMPLLGVVPDFNKMK

SEQ ID NO: 26 - protein, 229 aa, Streptococcus pneumoniae
MPTLEISQAKLELAKKTEEYYNALCTNPQLSGDDLKVFSISSVKAGEGKTTTSTNIAWAFAHAGYKTLLIDADMRNSVMSGVFKSRERITGLTEFLSGTTDLSQGLCDTNVENLFVIQAGSVSPNPIALLQSKNFSTMLGTLRKYFDYIVVDTAPIGIVIDAAIIMQKCDASILVTKAGETKRRELQKAKEQLEQTGKSCLGVVLNKFDTSVDKYGFYGSYGSYRKQKK

SEQ ID NO: 27 - protein, 453 aa, Streptococcus pneumoniae
MNEKLAKSSVAIVQSFLVILLTYLLSAVRETEIVSTTAIVLYILHYFVFYISDYGRNFFKRRYLIELVQTLKYILFFALAISISNFFLEDRFSISRRGMIYFLLLHVFLVYMLNLFIKWYWKRAYPNFKGSKKVFLLTATSHVEKVLDRLIESDDVVGELVAVSVLDKPDFQHDDLKVVAEGEIVNFATREVVDEVFINLPSEKYNIGELVSQFETMGIDVTVNLNAFDWARNKQICEMAGLNVVTFSTTFYKTSHVIAKRVIDIIGSLVGLILCGLVSIVLVPLIRKDGGSAIFAQTRIGKNGRHFTFYKFRSMCVDAEDKKRELMEQNTMQGGMFKVDDDPRITKIGHFIRKTSLDELPQFYNVLKGDMSLVGTRPPTVDEYEHYTPEQKRRLSFKPGITGLWQVSGRSEIKNFDEVVKLDVVYIDGWTIWKDIEILLKTVKVVLMKDGAK

SEQ ID NO: 28 - protein, 407 aa, Streptococcus pneumoniae
MERNSLLLFQTIRRKMKKSVYIIGSKGIPAKYGGFETFVEKLTEYQKDGNIQYYVACMRENSAKSGFTADTFEYNDAICYNIDVPNIGPARAIAYDIAAVNKAIEIAKKNKDEAPIFYILACRIGPFIARLKKKIQAIGGTLFVNPDGHEWLRAKWSLPVRKYWKFSEQLMVKYADLLVCDSKNIEKYIQNDYKQYQPKTTYIAYGTDTSPSILKSEDLKIRSWYQEKGLSENGYYLVVGRFVPENNYETMIREFIKSKSKKDFVLITNVEQNKFYDQLLQETGFDKDPRVKFVGTVYDQELLKYIRENAFAYFHGHEVGGTNPSLLEALASTKLNLLLDVGFNREVGEDGAIYWRKDNLHKVIEESEQKTIEEIKEIDILSTEQVEKRFTWDFIVNEYENLFLLGK

SEQ ID NO: 29 - protein, 395 aa, Streptococcus pneumoniae
MTIKINYMFFVCLSFFGIVLSSSQVIVNLGLSSIVQYIAYFLLLLCIFFTLIKNSPDVIANRIAYFSIISFLFIIGINLQNLPFSTKIYLSFSMLIISSLSTLPIKLINNINDFRRISYFLLNGILLSTFLGWLFNISLVTVAVEGIGFAYGFNGGLTHKNFYAITILVSYILLFISRKHGTKYQVDSLVLWFDLFLLLVSNTRTIYIILVVFWIVVHSGFIKYIKKNHRPVIITTWLVISLLSIIFFFKHIINNSESYTHRVLGIVNFFKYYESSKFHLFFGDAELAFGDMTKGYTHNIRSVLGWDGTVEMPLLSVMIKNGYVGLIGYGVVLFKFISSVLSMEDRRVKNIGLSILIPLLLSAMVENYIVNISFVFMPVCFCILCSIKNIEFKNN

SEQ ID NO: 30 - protein, 322 aa, Streptococcus pneumoniae
MKKVSIILPVYNVEQYIKKCLESIQQQTYPNLEVIIVNDGATDKSVEYCEQICKIDSRFSVTHKENGGLSDARNVGIDKAKGDYLIFVDSDDFVSQDMVSYLVSSMENNEADIAICDPAHYYSDRQNNDLNIFYPASSVKVYEKTEALCEMFYQKSFLVSAWAKIYKKELFDDIRFPVGKLFEDSAVMYLLFEKCEKIVYSNAKLYAYVHRDNSITTKKFSDKDLDILDISNTILDHYSGNFRVYKAAVSYKVSACFRILLNSSSEKKYNQIQKDCMTYILRNWRNMLFDKNVRLKNKLALISITLFNPFVKFIYSKVNRWE

SEQ ID NO: 31 - protein, 412 aa, Streptococcus pneumoniae
MNKYEERYQEDLSKNDFEKLINRRYLSDKELQVEYVKKGTVLPPKVFEMKLSNKLGLQKALHGKGGVVDSKGNYVELSEQKAVGMRNRVYGSYKFNHKNLAIRNEKVIYLNYFINQWGHFLLDVVGRLWYPLLKDTDTKLDYTCYAGTETKLEGNYLEFLELLGIDKSRLILINRPTQFSEIIIPESSILPGEYYTKEYKMLFNSLVANVKLDNNLESKKIYCSRARLDLAKGKEFGENGIEKVFLKNGYTPVYMETMSLKEQIRTLLSATTIVLTSGSLAHNLLFINNKINVFILNKTYRVNLHQFLINKISEASVSFVDIYRSPLPILYGYGPFLMDITKPLVNFFEDSGFTYDSGTILDKTDYFKFYLKWLWSYKFFLFRLNHIKEGNSEFEKSFKIIRRYYKMGRQYE

SEQ ID NO: 32 - protein, 462 aa, Streptococcus pneumoniae
MSKYKELAKNTGTFALANFSSKILIFLLVPIYTKVLTTTEYGFYDLVYTTIQLLVPILTLNISEAVMRFLMKEDVSKKSVFSIAILDIFLGSIIFCLLLLVNQIFSLSELISQYSIYIMAIFAFYTLNNFLIQYSKGIDKIGVTAISGVISAAVMLSMNILLLVVLNWGLLGFFIANICGYVIPCVYIIVKLKLWDLFELKIDRSLQWEMIYYTLPLILNTLSWWVNNTSDRYIITVIIGIQASAIISVAYKIPQIFSTISAIFIQSWQISAIKIQEEKEGNTFISKMLLYYNALLLIIASGIILFVKPISNILFGASFYSAWTLVPFLIISSLFNAISGYIGAIMGAKMDTKNIAKSALVGMIANVFLNIVLTFLMGLQGITISTMIASFLIFYMRKDSVEEIAPETYRAIYLSWFLLVVEASLLVYIDFIIGATLVTLINLFLLKDTLKPLCLKLLKGFK

SEQ ID NO: 33 - protein, 384 aa, Streptococcus pneumoniae
MKMNILQYIKILARTIFMLLISTVLLPVRLKNNKILFINFNGKGYGDNPKSICEYLRTTYPDLDLVWLARDNEGFPDGVRVVKYGTFQAFYEQASSKVWVYNVRAFARILKKRGQIYIQTWHGASSFKLIEKQADLPINYVLEAKYDARVTDIMISDSRKQTEEFQKYFWYSGEIFEVGMPRNDALFHYKEDYDKLNNIRKELSIHSDDYVILYAPTFRDDGDASYLDINFERLLQCVEHGIKKKCKFLIRLHPNHSHLCNNISFNKNIINATFYSDMQELTLLADVLVTDYSSSIFDFMLLNKPYVRYVNDLEKYAELRGVSDTYYELPDSIIKTAEELYDLLPKKIENFDYDSIKKYRNEILCPIFNGTASENVGRRIIQEL

SEQ ID NO: 34 - protein, 342 aa, Streptococcus pneumoniae; identical to SEQ ID NO: 16

SEQ ID NO: 35 - protein, 234 aa, Streptococcus pneumoniae; identical to SEQ ID NO: 17

SEQ ID NO: 36 - protein, 283 aa, Streptococcus pneumoniae
MNRIRRMKLTNRVDYFGADISELQNKKLFLFDMDGTIYEEDRLFEGTLELLDYIHNIGGEYIFITNNSSKSVVDYVEKVNRLGIKAERDNFFTSAQATIVYIKENYPKSKVYCQGTKSLIKELSDAGIDVTEQVSADIDVVLVGFDTELTSDKIRNTCEILSTKDVPFIATNPDIRCPVSFGFIPDCGSICDMISKSVDRKPVYIGKPEPTMVDIVRKKLNYSLFETVVIGDRLYTDIMTGINAGVTSVCVLTGEATVNDIQQDSIKPTYTFKNVKEMWKGIV

SEQ ID NO: 37 - protein, 289 aa, Streptococcus pneumoniae
MKGIILAGGSGTRLYPLTRAASKQLMPVYDKPMIYYPLSTLMLAGIRDILIISTPQDLPRFKELLQDGSEFGIKLSYAEQPSPDGLAQAFIIGEEFIGDDSVALILGDNIYHGPGLSTMLQKAAKKEKGATVFGYHVKDPERFGVVEFDENMNAISIEEKPEYPRSNYAVTGLYFYDNDVVEIAKSIKPSPRGELEITDVNKAYLDRGDLSVELMGRGFAWLDTGTHESLLEASQYIETVQRMQNVQVANLEEIAYRMGYISREDVLALAQPLKKNEYGQYLLRLIGEA

SEQ ID NO: 38 - protein, 197 aa, Streptococcus pneumoniae; identical to SEQ ID NO: 20

SEQ ID NO: 39 - protein, 349 aa, Streptococcus pneumoniae (
MTEYKNIIVTGGAGFIGSNFVHYVYENFPGVHVTVLDKLTYAGNRANIEEILGNRVELVVGDIADAELVDKLAAQADAIVHYAAESHNDNSLNDPSPFIHTNFIGTYTLLEAARKYDIRFHHVSTDEVYGDLPLREDLPGHGEGPGEKFTAETKYNPSSPYSSTKAASDLIVKAWVRSFGVKATISNCSNNYGPYQHIEKFIPRQITNILSGIKPKLYGEGKNVRDWIHTNDHSSGVWTILTKGQIGETYLIGADGEKNNKEVLELILKEMGQATDAYDHVTDRAGHDLRYAIDASKLRDELGWKPEFTNFEAGLKATIKWYTDNQEWWKAEKEAVEANYAKTQEIITV

SEQ ID NO: 40 - protein, 283 aa, Streptococcus pneumoniae
MILITGANGQLGTELRYLLDERNEEYVAVDVAEMDITNEEMVEKVFEEVKPTLVYHCAAYTAVDAAEDEGKELNFAINVTGTKNVAKASEKHGATLVYISTDYVFDGKKPVGQEWEVDDRPDPQTEYGRTKRMGEELVEKHVSNFYIIRTAWVFGNYGKNFVFTMQNLAKTHKTLTVVNDQYGRPTWTRTLAEFMTYLAENRKEFGYYHLSNDATEDTTWYDFAVEILKDTDVEVKPVDSSQFPAKAKRPLNSTMSLAKAKATGFVIPTWQDALQEFYKQEVR

SEQ ID NO: 41 - protein, 481 aa, Streptococcus pneumoniae
MSRRFKKSRSQKVKRSVNIVLLTIYLLLVCFLLFLIFKYNILAFRYLNLVVTALVLLVALVGLLLIIYKKAEKFTIFLLVFSILVSSVSLFAVQQFVGLTNRLNATSNYSEYSISVAVLADSDIENVTQLTSVTAPTGTDNENIQKLLADIKSSQNTDLTVDQSSSYLAAYKSLIAGETKAIVLNSVFENIIESEYPDYASKIKKIYTKGFTKKVEAPKTSKNQSFNIYVSGIDTYGPISSVSRSDVNILMTVNRDTKKILLTTTPRDAYVPIADGGNNQKDKLTHAGIYGVDSSIHTLENLYGVDINYYVRLNFTSFLKMIDLLGGVDVHNDQEFSALHGKFHFPVGNVHLDSEQALGFVRERYSLADGDRDRGRNQQKVIVAILQKLTSTEALKNYSTIIDSLQDSIQTNMPLETMINLVNAQLESGGNYKVNSQDLKGTGRTDLPSYAMPDSNLYVMEIDDSSLAVVKAAIQDVMEGR

SEQ ID NO: 42 - protein, 243 aa, Streptococcus pneumoniae
MIDIHSHIVFDVDDGPKSREESKALLTESYRQGVRTIVSTSHRRKGMFETPEEKIAENFLQVREIAKEVADDLVIAYGAEIYYTLDALEKLEKKEIPTLNDSRYALIEFSMNTPYRDIHSALSKILMLGITPVIAHIERYDALENNEKRVRELIDMGCYTQVNSSHVLKPKLFGERYKFMKKRAQYFLEQDLVHVIASDMHNLDGRPPHMAEAYDLVTQKYGEAKAQELFIDNPRKIVMDQLI

SEQ ID NO: 43 - protein, 231 aa, Streptococcus pneumoniae
MMKEQNTIEIDVFQLFKTLWKRKLMILIVALVTGTGAFAYSTFIVKPEYTSTTRIYVVNRNQGDKPGLTNQDLQAGTYLVKDYREIILSQDALEKVATNLKLDMPAKTLASKVQVAVPADTRIVSISVKDKQPEEASRIANSLREVAAEKIVAVTRVSDVTTLEEARPATTPSSPNVRRNSLFGFLGGAVVTVIAVLLIELLDTRVKRPEDVEDVLKIPLLGLVPDFDKIK

SEQ ID NO: 44 - protein, 229 aa, Streptococcus pneumoniae
MPTLEISQAKLDSVKKAEEYYNALCTNLQLSGDGLKVFSITSVKIGEGKSTTSANIAWAFARAGYKTLLIDGDIRNSVMLGVFKARNKITGLTEFLSGTTDLSQGLCDTNIENLFVIQAGSVSPNPTALLQSKNFTTMLETLRKYFDYIIVDTAPVGVVIDAAIITRNCDASILVTEAGEINRRDIQKAKEQLEHTGKPFLGIVLNKFDTSVDKYGSYGNYGNYGKNKK

SEQ ID NO: 45 - protein, 455 aa, Streptococcus pneumoniae
MNEKILRSSLAIIQSFLVILLTYLLSAVRETEIVSTTAIALCILHYFVFYISDYGQDFFKRRYLIELVQTLKYILFFALAIGISNFFLEDRFSISRRGMIYFLTLHALLVYVLNLFIKWYWKRAYPNFKGSKKILLLTATSRVEKVLDRLIESNEVVGKLVAVSVLDKPDFQHDCLKVVAEGGIVNFATHEVVDEVFINLPSEKYNIGELVSQFETMGIDVIVNLNAFDRSLARNKQIREMAGLNVVTFSTTFYKTSHVIAKRIIDIVGALVGLILCGLVSIVLVPLIRKDGGSAIFAQTRIGKNGRQFTFYKFRSMCVDAEAKKRELMEQNTMQGGMFKVDDDPRITKIGCFIRKTSLDELPQFYNVLKGDMSLVGTRPPTVDEYEHYTPEQKRRLSFKPGITGLWQVSGRSEIKNFDEVVKLDVAYIDGWTIWKDIEILLKTVKVVFMRDGAK

SEQ ID NO: 46 - protein, 392 aa, Streptococcus pneumoniae
MKKSVYIIGSKGIPAKYGGFETFVEKLTAFQQDKAIQYYVACMRENSAKSGTTEDVFEHNGAICYNVDVPNFGPARAIAYDIAAINRAIEIAKENKDEDPIFYILACRIGPFIHGIKKKIQEIGGTLLVNPDGHEWLRAKWSAPVRRYWKISEGLMVKHADLLVCDSKNIEKYIQEDYKQYQPKTTYIAYGTDTTRSVLKSSDEKVRSWFKEKNVSENEYYLVVGRFVPENNYESMIRGFLASNSKKDFVLITNVEQNKFYNQLLAKTGFDKDPRVKFVGTVYEQELLKYIRENAFAYFHGHEVGGTNPSLLEALASTKLNLLLDVGFNREVAEDGAIYWKKDNLHEIIETSEQKTQKEIDEKDILSIKQVTERFSWELIVNEYEKLFLCEK

SEQ ID NO: 47 - protein, 397 aa, Streptococcus pneumoniae
MTIKINNLFFVCLSFFGIVLSSSQVIVNLGLSSIIQYISYFMLMLCVFLTLIKNTLNVFANRIIYFLIISFLFIIGINLQNLPLSRKIYLSFSMLIISSLSTLPIKLINNLSDLRRISYYLLHSIFLSVFLGLVFKISLVTVAVEGIGFSYGFNGGLTHKNFYAITILVSYILLYVSRKYDAKHQIDSFVLWLDLFLLLISNTRTVYIILVVFWIIINRNFINNIKKEHRLVVTATTIVISLLALTFFFKHIINNSESYSHRVLGVVNFFKYYESDRFHLFFGDAELAFGNTTKGYGHNIRSVLGWDGTVEMPLLSVMIKNGYVGLVGYIIVLFKFISSIISVKNSTKKNIGLSIFIPLLLSATVENYIVNISFVFMPVCFCILCSIKNIKLVNNRK

SEQ ID NO: 48 - protein, 323 aa, Streptococcus pneumoniae
MEKLVSIILPVYNVEQYIKNCLESIQQQTYSNLEVIIVNDGSTDKSVEYCEQICKIDSRFSITHKENGGLSDARNVGIDKSKGDYLIFVDSDDFVSQDMVSYLVSCMENNEADIAICDPVHYYSDRQNNDLNIFSPASNVKVYETTEALCEMFYQKSFLVSAWAKIFKRELFDDIRFPVGKLFEDSAIMYLLFEKCETIAYSDAELYAYVHRDNSITTKKFSDRDLDILEITNTIINHYGDNLRVYTAAVSYKVSACFRILLNSPSGEKYKKVQKECLSYILQNWRNILFNNNVRLKNKLALISITIFNPFVKFIYSKVNRWE

SEQ ID NO: 49 - protein, 410 aa, Streptococcus pneumoniae; identical to SEQ ID NO: 13

SEQ ID NO: 50 - protein, 461 aa, Streptococcus pneumoniae
MSKYKELAKNTGIFALANFSSKILIFLLVPIYTRVLTTTEYGFYDLVYTTIQLFVPILTLNISEAVMRFLMKDGVSKKSVFSIAVLDIFIGSIAFALLLLVNNLFSLSDLISQYSIYIFVIFVFYTLNNFLIQFSKGIDKIGVTAISGVISTAVMLAMNVILLVVFDWGLLGFFIANVCGYVIPCIYIVSRLRLWELFEIKIDKKLQWEMVYYALPLVLNILSWWVNNTSDRYIVTAIVGIQASAIISVAYKIPQILSTISAIFIQSWQISAIKIQEDKSDTTFVSNMLLYYNALLLIIASGIILFVKPISNILFGISFYSAWELVPFLIISSLFNAISGCIGAIMGAKMDTHNIAKSALVGMIANIILNIVLTFLMGPQGITISTLIASFLIFYMRKDSVKEINSETYRAIYLSWILLVVEACLLIYMDFIIGALIAMVINLFLLKDVIKPLYLKIFKRN

SEQ ID NO: 51 - protein, 382 aa, Streptococcus pneumoniae; identical to SEQ ID NO: 15

SEQ ID NO: 52 - protein, 342 aa, Streptococcus pneumoniae; identical to SEQ ID NO: 16

SEQ ID NO: 53 - protein, 234 aa, Streptococcus pneumoniae; identical to SEQ ID NO: 17

SEQ ID NO: 54 - protein, 277 aa, Streptococcus pneumoniae; identical to SEQ ID NO: 18

SEQ ID NO: 55 - protein, 289 aa, Streptococcus pneumoniae; identical to SEQ ID NO: 19

SEQ ID NO: 56 - protein, 197 aa, Streptococcus pneumoniae; identical to SEQ ID NO: 20

SEQ ID NO: 57 - protein, 349 aa, Streptococcus pneumoniae; identical to SEQ ID NO: 21

SEQ ID NO: 58 - protein, 283 aa, Streptococcus pneumoniae; identical to SEQ ID NO: 22

SEQ ID NO: 59 - protein, 358 aa, E. coli
MEENNMKTVAVVGTVGVPACYGGFESLVQNLIDYQSDGIQYQIFCSSKKYDKKFKNYKNAELIYLPINANGVSSIIYDIMCLIICLFKRPDVVLILGVSGCLFLPIYKLFSKSKIIVNIDGLEWRRNKWGTFAKKFLKISEAISIRIADIIISDNQAIADYVENKYKKKSVVIAYGGDHATNLSTPIDNDQKKEGYYLGLCRIEPENNIEMILNAFINTDKKIKFMGNWDNSEYGRQLKKYYSNYPNITLLEPNYNIEELYKLRKNCLAYIHGHSAGGTNPSLVEAMHFNIPIFAFDCDFNRYTTNNLAHYFNDSEQLSLLAESLSFGNLKCRVLDLKNYAEDMYNWRHIAAMYESIY

SEQ ID NO: 60 - protein, 360 aa, E. coli
MTEQFSEKKIDVVGIVGLPACYGGFESLVQNLVDYQSQNIKYNVYCSRKKYKNTPKKYKRADLKYIPFDANGSSSILYDIYSLFLSLFNKVDVVLILGVSGCVFLPIYRFFSSSKVIVNIDGLEWKRAKWKGIAKWYLKISEKIAVKYSDVVVADNEAIAKYVLKKYGLEAKIIAYGGDHSLVKKPISVIKEDYFFTVCRIEPENNIRMILEAFKNTTHSLKIVGNWDSSLYGRRLKEEFGNYNNIEIIDPIYDSDILFNFRSLCRGYIHGHSAGGTNPSLVEAMHFQIPIIAFDCDFNRFTTDNYAFYFKNKNELSFIVNDILNGNQNEQAEICAKKMKEIATKKYTWDTIAKMYEELY

SEQ ID NO: 61 - protein, 351 aa, Cronobacter sakazakii
MKRIAVVGTVGIPACYGGFESLVENLTKYKGAGYQYYIFCSSKNYPEKSDSHNDAQLIYVPLKANGIQSILYDIVSLWKCLFLKVDTILILGVSGCIFLPVFRLLSNAKIITNIDGLEWKREKWNYPIKKFLKFSELLAVKYSHAIVTDNRAITDYVKKEYNVSSFTIAYGGDHAVRPSNNNNNIKSSYALGLCRIEPENNVELILKAFTLSEDKLKFVGNWNASSYGRMLKKNYSNYSNIELIEPIYDIDKLYILRSGCDKYIHGHSAGGTNPSLVEMMHFGVPIFAFDCEFNRHSTDNKAFYFKDAQHLADLVKMKDNTELEKNSCNMKVLAQENYTWQKITASYESLY

SEQ ID NO: 62 - protein, 664 aa, Campylobacter jejuni
IISNDGYAFAEGARDMIAGFHQPNDLSYYGSSLSTLTYWLYKITPFSFESIILYMSTFLSSLVVIPIILLANEYKRPLMGFVAALLASIANSYYNRTMSGYYDTDMLVIVLPMFILFFMVRMILKKDFFSLIALPLFIGIYLWWYPSSYTLNVALIGLFLIYTLIFHRKEKIFYIAVILSSLTLSNIAWFYQSTIIVILFALFALEQKRLNFVIIGILASVTLIFLILSGGVDPILYQLKFYIFRSDESANLTQGFMYFNVNQTIQEVENVDLSEFMRRISGSEIVFLFSLFGFVWLLRKHKSMIMALPILVLGFLALKGGLRFTIYSVPVMALGFGFLLSEFKAILVKKYSQLTSNVCIVFATILTLAPVFIHIYNYKAPTVFSQNEASLLNQLKNIANREDYVVTWWDYGYPVRYYSDVKTLVDGGKHLGKDNFFPSFALSKDEQAAANMARLSVEYTEKSFYAPQNDILKTDILQAMMKDYNQSNVDLFLASLSKPDFKIDTPKTRDIYLYMPARMSLIFSTVASFSFINLDTGVLDKPFTFSTAYPLDVKNGEIYLSNGVVLSDDFRSFKIGDNVVSVNSIVEINSIKQGEYKITPIDDKAQFYIFYLKDSAIPYAQFILMDKTMFNSAYVQMFFLGNYDKNLFDLVINSRDAKVFKLKI

SEQ ID NO: 63 - protein, 257 aa, E. coli
MMVFGKLYLSSLGYIFGSWEMVLGPFGYFLTLFAVWAAINAFNMVDGIDGLLGGLSCVSFAAIGMILWFDGQTSLAIWCFAMIAAILPYIMLNLGILGRRYKVFMGDAGSTLIGFTVIWILLETTQGKTHPISPVTALWIIAIPLMDMVAIMYRRLRKGMSPFSPDRQHIHHLIMRAGFTSRQAFVLITLAAALLASIGVLAEYSHFVPEWVMLVLFLLAFFLYGYCIKRAWKVARFIKRVKRRLRRNRGGSPNLTK

SEQ ID NO: 64 - protein, 207 aa, E. coli
MSTIIMDLCSYTRLGLTGYLLSRGVKKREINDIETVDDLAIACDSQRPSVVFINEDCFIHDASNSQRIKLIINQHPNTLFIVFMAIANVHFDEYLLVRKNLLISSKSIKPESLDDILGDILKKETTITSFLNMPTLSLSRTESSMLRMWMAGQGTIQISDQMNIKAKTVSSHKGNIKRKIKTHNKQVIYHVVRLTDNVTNGIFVNMR

SEQ ID NO: 65 - protein, 713 aa, Campylobacter jejuni
MLKKEYLKNPYLVLFAMIILAYVFSVFCRFYWVWWASEFNEYFFNNQLMIISNDGYAFAEGARDMIAGFHQPNDLSYYGSSLSALTYWLYKITPFSFESIILYMSTFLSSLVVIPTILLANEYKRPLMGFAAALLASIANSYYNRTMSGYYDTDMLVIVLPMFILFFMVRMILKKDFFSLIALPLFIGIYLWWYPSSYTLNVALIGLFLIYTLIFHRKEKIFYIAVILSSLTLSNIAWFYQSAIIVILFALFALEQKRLNFMIIGILGSATLIFLILSGGVDPILYQLKFYIFRSDESANLTQGFMYFNVNQTIQEVENVDLSEFMRRISGSEIVFLFSLFGFVWLLRKHKSMIMALPILVLGFLALKGGLRFTIYSVPVMALGFGFLLSEFKAIMVKKYSQLTSNVCIVFATILTLAPVFIHIYNYKAPTVFSQNEASLLNQLKNIANREDYVVTWWDYGYPVRYYSDVKTLVDGGKHLGKDNFFPSFALSKDEQAAANMARLSVEYTEKSFYAPQNDILKTDILQAMMKDYNQSNVDLFLASLSKPDFKIDTPKTRDIYLYMPARMSLIFSTVASFSFINLDTGVLDKPFTFSTAYPLDVKNGEIYLSNGVVLSDDFRSFKIGDNVVSVNSIVEINSIKQGEYKITPIDDKAQFYIFYLKDSAIPYAQFILMDKTMFNSAYVQMFFLGNYDKNLFDLVINSRDAKVFKLKI

SEQ ID NO: 66 - protein, 378 aa, Salmonella typhimurium
MPSLNVKQEKNQSFAGYSLPPANSHEIDLFSLIEVLWQAKRRILATVFAFACVGLLLSFLLPQKWTSQAIVTPAESVQWQGLERTLTALRVLDMEVSVDRGSVFNLFIKKFSSPSLLEEYLRSSPYVMDQLKGAQIDEQDLHRAIVLLSEKMKAVDSNVGKKNETSLFTSWTLSFTAPTREEAQKVLAGYIQYISDIVVKETLENIRNQLEIKTRYEQEKLAMDRVRLKNQLDANIQRLHYSLEIANAAGIKRPVYSNGQAVKDDPDFSISLGADGISRKLEIEKGVTDVAEIDGDLRNRQYHVEQLAAMNVSDVKFTPFKYQLSPSLPVKKDGPGKAIIIILAALIGGMMACGGVLLRHAMVSRKMENALAIDERLV